European Patent Application EP 4 703 380 A1, published March 4, 2026. Title: Integrin-targeting antibodies and uses thereof. Applicant: NIO BIOPHARMACEUTICALS. INC. The sequence listing filed with the application follows.

SEQUENCE LISTING (47 sequences)

SEQ ID NO: 1 - protein, 5 aa, synthetic construct
  REGION 1..5: note = VH CDR1
TYWMN

SEQ ID NO: 2 - protein, 5 aa, synthetic construct
  REGION 1..5: note = VH CDR1
DHYMS

SEQ ID NO: 3 - protein, 6 aa, synthetic construct
  REGION 1..6: note = VH CDR1
SSYYWS

SEQ ID NO: 4 - protein, 5 aa, synthetic construct
  REGION 1..5: note = VH CDR1
DYHWS

SEQ ID NO: 5 - protein, 17 aa, synthetic construct
  REGION 1..17: note = VH CDR2
AISGSGGSTYYADSVKG

SEQ ID NO: 6 - protein, 17 aa, synthetic construct
  REGION 1..17: note = VH CDR2
YISNRGYTIHYADFVKG

SEQ ID NO: 7 - protein, 15 aa, synthetic construct
  REGION 1..15: note = VH CDR2
YIYDTVTDYNPSLKS

SEQ ID NO: 8 - protein, 16 aa, synthetic construct
  REGION 1..16: note = VH CDR2
FISPSAINNYNPSLKS

SEQ ID NO: 9 - protein, 9 aa, synthetic construct
  REGION 1..9: note = VH CDR3
DQGYLPFDY

SEQ ID NO: 10 - protein, 10 aa, synthetic construct
  REGION 1..10: note = VH CDR3
DRGTIDAFDL

SEQ ID NO: 11 - protein, 10 aa, synthetic construct
  REGION 1..10: note = VH CDR3
ETGSWYTFDY

SEQ ID NO: 12 - protein, 7 aa, synthetic construct
  REGION 1..7: note = VH CDR3
GGWSLDS

SEQ ID NO: 13 - protein, 11 aa, synthetic construct
  REGION 1..11: note = VL CDR1
RASQDIGNDLG

SEQ ID NO: 14 - protein, 14 aa, synthetic construct
  REGION 1..14: note = VL CDR1
SGTSDDIGRYNYVS

SEQ ID NO: 15 - protein, 11 aa, synthetic construct
  REGION 1..11: note = VL CDR1
RATQDIDNFLN

SEQ ID NO: 16 - protein, 11 aa, synthetic construct
  REGION 1..11: note = VL CDR1
QASQDITDFLN

SEQ ID NO: 17 - protein, 7 aa, synthetic construct
  REGION 1..7: note = VL CDR2
GASSLQS

SEQ ID NO: 18 - protein, 7 aa, synthetic construct
  REGION 1..7: note = VL CDR2
DVTRRSS

SEQ ID NO: 19 - protein, 7 aa, synthetic construct
  REGION 1..7: note = VL CDR2
EASNLET

SEQ ID NO: 20 - protein, 7 aa, synthetic construct
  REGION 1..7: note = VL CDR2
DASNLET

SEQ ID NO: 21 - protein, 9 aa, synthetic construct
  REGION 1..9: note = VL CDR3
LQDYSYPLT

SEQ ID NO: 22 - protein, 10 aa, synthetic construct
  REGION 1..10: note = VL CDR3
SSFTNNRTVV

SEQ ID NO: 23 - protein, 9 aa, synthetic construct
  REGION 1..9: note = VL CDR3
QQSYSSPYS

SEQ ID NO: 24 - protein, 9 aa, synthetic construct
  REGION 1..9: note = VL CDR3
QQSYTTPYS

SEQ ID NO: 25 - protein, 118 aa, synthetic construct
  REGION 1..118: note = Heavy chain variable region
QVQLVQSGGGLVQPGESLRLSCAASGFSIGTYWMNWVRQAPGKGLEWVSAISGSGGSTYYADSVKGRFTISRDNSKNTLYLQMNSLRAEDTAVYYCARDQGYLPFDYWGLGTLVTVSS

SEQ ID NO: 26 - protein, 120 aa, synthetic construct
  REGION 1..120: note = Heavy chain variable region
QVQLVQSGGGLVNPGGSLRLSCAASGFPFSDHYMSWIRQAPGKGLEWVSYISNRGYTIHYADFVKGRFTISRDNAENTLYLQMNSLRAEDTAVYYCARDRGTIDAFDLWGQGTMVTVSSG

SEQ ID NO: 27 - protein, 117 aa, synthetic construct
  REGION 1..117: note = Heavy chain variable region
QVQLQESGPRQVKPSETLSLTCTVTGGSMSSYYWSWIRQSPGKGLEWIGYIYDTVTDYNPSLKSRVTISVDTSKNQFSLKLTSVTAVDTAVYYCARETGSWYTFDYWSPGALVTVSS

SEQ ID NO: 28 - protein, 115 aa, synthetic construct
  REGION 1..115: note = Heavy chain variable region
QVQLQESGPGLVKPSETLSLTCSVSGGSISDYHWSWIRQFPGKGLEWIGFISPSAINNYNPSLKSRVSMSTDTSKNQFSLTLTSVTAVDTAVYYCARGGWSLDSWGQGTLVTVSS

SEQ ID NO: 29 - protein, 108 aa, synthetic construct
  REGION 1..108: note = Light chain variable region
DIQMTQSPSSLSASVGDRVTITCRASQDIGNDLGWYQQKPGKAPKLLIYGASSLQSGVPSRFSGRRSATDFTLTIFNLQAEDFASYYCLQDYSYPLTFGGGTKVEIKR

SEQ ID NO: 30 - protein, 111 aa, synthetic construct
  REGION 1..111: note = Light chain variable region
QSALTQPASVSGSPGQSITIPCSGTSDDIGRYNYVSWYQQHPGKAPKLLIYDVTRRSSGVSSHFSGSKSGSTASLIISGLQADDEADYFCSSFTNNRTVVFGGGTKLTVLG

SEQ ID NO: 31 - protein, 108 aa, synthetic construct
  REGION 1..108: note = Light chain variable region
DIQMTQSPSSLSASVGDRVTITCRATQDIDNFLNWYQQKPGKAPKLLIYEASNLETGVPSRFSGSGSGTDFTLTISSLQPDDFALYYCQQSYSSPYSFGPGTKVDIKR

SEQ ID NO: 32 - protein, 108 aa, synthetic construct
  REGION 1..108: note = Light chain variable region
DIQMTQSPSSLSASVGDRVTITCQASQDITDFLNWYQQKPGRAPKLLIYDASNLETGVPSRFSGSGSGTDFTLTISGLQPDDFALYYCQQSYTTPYSFGPGTKVEIKR

SEQ ID NO: 33 - protein, 5 aa, synthetic construct
  REGION 1..5: note = peptide linker
GGGGS

SEQ ID NO: 34 - protein, 10 aa, synthetic construct
  REGION 1..10: note = peptide linker
GGGGSGGGGS

SEQ ID NO: 35 - protein, 10 aa, synthetic construct
  REGION 1..10: note = peptide linker
SGGGGSGGGG

SEQ ID NO: 36 - protein, 14 aa, synthetic construct
  REGION 1..14: note = peptide linker
GGGGSGGGGSGGGG

SEQ ID NO: 37 - protein, 10 aa, synthetic construct
  REGION 1..10: note = peptide linker
GSPGSSSSGS

SEQ ID NO: 38 - protein, 15 aa, synthetic construct
  REGION 1..15: note = peptide linker
GGGGSGGGGSGGGGS

SEQ ID NO: 39 - protein, 8 aa, synthetic construct
  REGION 1..8: note = peptide linker
GSGSGSGS

SEQ ID NO: 40 - protein, 8 aa, synthetic construct
  REGION 1..8: note = peptide linker
GSGSGNGS

SEQ ID NO: 41 - protein, 8 aa, synthetic construct
  REGION 1..8: note = peptide linker
GGSGSGSG

SEQ ID NO: 42 - protein, 6 aa, synthetic construct
  REGION 1..6: note = peptide linker
GGSGSG

SEQ ID NO: 43 - protein, 4 aa, synthetic construct
  REGION 1..4: note = peptide linker
GGSG

SEQ ID NO: 44 - protein, 8 aa, synthetic construct
  REGION 1..8: note = peptide linker
GGSGNGSG

SEQ ID NO: 45 - protein, 8 aa, synthetic construct
  REGION 1..8: note = peptide linker
GGNGSGSG

SEQ ID NO: 46 - protein, 6 aa, synthetic construct
  REGION 1..6: note = peptide linker
GGNGSG

SEQ ID NO: 47 - protein, 15 aa, synthetic construct
  REGION 1..15: note = peptide linker
GGGGSGGGSCGGGGS